European Patent Application EP 4 725 555 A2, published April 15, 2026. Title: SINGLE-DOMAIN 4-1BB ANTIBODIES. Applicant: Concept to Medicine Biotech Co., Ltd. Application WO. The sequence listing filed with the application follows.

SEQUENCE LISTING (44 sequences)

SEQ ID NO: 1 - protein, 115 aa, synthetic construct
QVQLVESGGGLVQAGGSLRLSCAASGDIFSIMFWYRQPQGKQREYVAHITSNGRTNYADSVTGRFTISRGNNDNTMYLQMDNLKPQDTAVYYCAADDATNTRTYWGQGTQVTVSS

SEQ ID NO: 2 - protein, 126 aa, synthetic construct
QVQLVESGGGLVQPGGSLRLSCAASGFTLDYYAIGWFRQAPGKEREGVSCISSSDGSTYYADSVKGRFTISRDNAKNTVYLQMNSLKPEDTAVYYCATDTTTRCPIWSYYVESDYWGQGTQVTVSS

SEQ ID NO: 3 - protein, 126 aa, synthetic construct
QVQLVESGGGLVQPGGSLRLSCAASGFAFSDYAIGWFRQAPGKEREGVSCISSSDGSTYYADSVKGRFTISRDNAKNTVYLQMNSLKPEDTAVYYCATDTTTRCPIWSYYVESDYWGQGTQVTVSS

SEQ ID NO: 4 - protein, 116 aa, synthetic construct
EVQLVESGGGLVQAGGSLRLSCAASGSIFSYMFWYRQPQGKQREYVAHITSGGRTNYADSVTGRFTISRGNNDNTMYLQMNNLKPEDTAVYYCAADDAVYTDRTYWGQGTQVTVSS

SEQ ID NO: 5 - protein, 126 aa, synthetic construct
EVQLVESGGGLVQPGGSLRLSCAASGLSLDYYAIGWFRQAPGKEREGVSCISSSGRSTNYADSVKGRFTISRDNAKNTVYLQMNSLKPEDTADYYCATDTTTRCPIWSNYVESDYWGQGTQVTVSS

SEQ ID NO: 6 - protein, 4 aa, synthetic construct
SIMF

SEQ ID NO: 7 - protein, 16 aa, synthetic construct
HITSNGRTNYADSVTG

SEQ ID NO: 8 - protein, 9 aa, synthetic construct
DDATNTRTY

SEQ ID NO: 9 - protein, 5 aa, synthetic construct
YYAIG

SEQ ID NO: 10 - protein, 17 aa, synthetic construct
CISSSDGSTYYADSVKG

SEQ ID NO: 11 - protein, 17 aa, synthetic construct
DTTTRCPIWSYYVESDY

SEQ ID NO: 12 - protein, 5 aa, synthetic construct
DYAIG

SEQ ID NO: 13 - protein, 17 aa, synthetic construct
CISSSDGSTYYADSVKG

SEQ ID NO: 14 - protein, 17 aa, synthetic construct
DTTTRCPIWSYYVESDY

SEQ ID NO: 15 - protein, 4 aa, synthetic construct
SYMF

SEQ ID NO: 16 - protein, 16 aa, synthetic construct
HITSGGRTNYADSVTG

SEQ ID NO: 17 - protein, 10 aa, synthetic construct
DDAVYTDRTY

SEQ ID NO: 18 - protein, 5 aa, synthetic construct
YYAIG

SEQ ID NO: 19 - protein, 17 aa, synthetic construct
CISSSGRSTNYADSVKG

SEQ ID NO: 20 - protein, 17 aa, synthetic construct
DTTTRCPIWSNYVESDY

SEQ ID NO: 21 - protein, 115 aa, synthetic construct
QVQLVESGGGLVQPGGSLRLSCSASGDIFSIMFWYRQAPGKQREYVSHITSNGRTNYADSVTGRFTISRDNSKNTLYLQMNSLRAEDTAVYYCAADDATNTRTYWGQGTLVTVSS

SEQ ID NO: 22 - protein, 115 aa, synthetic construct
QVQLVESGGGLVQPGGSLRLSCAASGDIFSIMFWYRQAPGKQREYVAHITSNGRTNYADSVTGRFTISRDNNKNTLYLQMNSLRAEDTAVYYCAADDATNTRTYWGQGTLVTVSS

SEQ ID NO: 23 - protein, 115 aa, synthetic construct
QVQLVESGGGLVQPGGSLRLSCAASGDIFSIMFWYRQAPGKQREYVAHITSNGRTNYADSVTGRFTISRDNSKNTMYLQMDSLRAEDTAVYYCAADDATNTRTYWGQGTLVTVSS

SEQ ID NO: 24 - protein, 115 aa, synthetic construct
QVQLVESGGGLVQPGGSLRLSCAASGDIFSIMFWYRQPQGKQREYVAHITSNGRTNYADSVTGRFTISRDNNKNTLYLQMDSLRAEDTAVYYCAADDATNTRTYWGQGTLVTVSS

SEQ ID NO: 25 - protein, 115 aa, synthetic construct
QVQLVESGGGLVQPGGSLRLSCSASGDIFSIMFWYRQAPGKQREYVAHITSNGRTNYADSVTGRFTISRDNSKNTLYLQMNSLRAEDTAVYYCARDDATNTRTYWGQGTLVTVSS

SEQ ID NO: 26 - protein, 126 aa, synthetic construct
EVQLVESGGGLVQPGGSLRLSCAASGFAFSDYAIGWVRQAPGKGLEWVSCISSSDGSTYYADSVKGRFTISRDNSKNTLYLQMNSLRAEDTAVYYCAKDTTTRCPIWSYYVESDYWGQGTLVTVSS

SEQ ID NO: 27 - protein, 126 aa, synthetic construct
EVQLVESGGGLVQPGGSLRLSCAASGFAFSDYAIGWFRQAPGKEREGVSCISSSDGSTYYADSVKGRFTISRDNSKNTLYLQMNSLRAEDTAVYYCATDTTTRCPIWSYYVESDYWGQGTLVTVSS

SEQ ID NO: 28 - protein, 126 aa, synthetic construct
EVQLVESGGGLVQPGGSLRLSCAASGFAFSDYAIGWFRQAPGKEREGVSCISSSDGSTYYADSVKGRFTISRDNAKNTLYLQMNSLRAEDTAVYYCAKDTTTRCPIWSYYVESDYWGQGTLVTVSS

SEQ ID NO: 29 - protein, 126 aa, synthetic construct
EVQLVESGGGLVQPGGSLRLSCAASGFAFSDYAIGWFRQAPGKEREGVSCISSSDGSTYYADSVKGRFTISRDNAKNTLYLQMNSLRAEDTAVYYCATDTTTRCPIWSYYVESDYWGQGTLVTVSS

SEQ ID NO: 30 - protein, 126 aa, synthetic construct
EVQLVESGGGLVQPGGSLRLSCAASGFAFSDYAIGWFRQAPGKEREGVSCISSSDGSTYYADSVKGRFTISRDNAKNTLYLQMNSLRPEDTAVYYCATDTTTRCPIWSYYVESDYWGQGTLVTVSS

SEQ ID NO: 31 - protein, 126 aa, synthetic construct
EVQLVESGGGLVQPGGSLRLSCAASGFTFSYYAIGWVRQAPGKGLEWVSCISSSDGSTYYADSVKGRFTISRDNSKNTLYLQMNSLRAEDTAVYYCAKDTTTRCPIWSYYVESDYWGQGTLVTVSS

SEQ ID NO: 32 - protein, 126 aa, synthetic construct
EVQLVESGGGLVQPGGSLRLSCAASGFTFSYYAIGWFRQAPGKEREGVSCISSSDGSTYYADSVKGRFTISRDNSKNTLYLQMNSLRAEDTAVYYCATDTTTRCPIWSYYVESDYWGQGTLVTVSS

SEQ ID NO: 33 - protein, 126 aa, synthetic construct
EVQLVESGGGLVQPGGSLRLSCAASGFTLDYYAIGWFRQAPGKEREGVSCISSSDGSTYYADSVKGRFTISRDNSKNTLYLQMNSLRAEDTAVYYCATDTTTRCPIWSYYVESDYWGQGTLVTVSS

SEQ ID NO: 34 - protein, 126 aa, synthetic construct
EVQLVESGGGLVQPGGSLRLSCAASGFTLDYYAIGWFRQAPGKEREGVSCISSSDGSTYYADSVKGRFTISRDNAKNTLYLQMNSLRPEDTAVYYCATDTTTRCPIWSYYVESDYWGQGTLVTVSS

SEQ ID NO: 35 - protein, 126 aa, synthetic construct
EVQLVESGGGLVQPGGSLRLSCAASGFTFSYYAIGWVRQAPGKGLEWVSCISSSGRSTNYADSVKGRFTISRDNSKNTLYLQMNSLRAEDTAVYYCAKDTTTRCPIWSNYVESDYWGQGTLVTVSS

SEQ ID NO: 36 - protein, 126 aa, synthetic construct
EVQLVESGGGLVQPGGSLRLSCAASGFTFSYYAIGWFRQAPGKEREGVSCISSSGRSTNYADSVKGRFTISRDNSKNTLYLQMNSLRAEDTAVYYCATDTTTRCPIWSNYVESDYWGQGTLVTVSS

SEQ ID NO: 37 - protein, 126 aa, synthetic construct
EVQLVESGGGLVQPGGSLRLSCAASGLTFSYYAIGWFRQAPGKEREGVSCISSSGRSTNYADSVKGRFTISRDNSKNTLYLQMNSLRAEDTAVYYCATDTTTRCPIWSNYVESDYWGQGTLVTVSS

SEQ ID NO: 38 - protein, 126 aa, synthetic construct
EVQLVESGGGLVQPGGSLRLSCAASGLTLSYYAIGWFRQAPGKEREGVSCISSSGRSTNYADSVKGRFTISRDNSKNTLYLQMNSLRAEDTADYYCATDTTTRCPIWSNYVESDYWGQGTLVTVSS

SEQ ID NO: 39 - protein, 16 aa, synthetic construct
HITSNARTNYADSVTG

SEQ ID NO: 40 - protein, 16 aa, synthetic construct
HITSQGRTNYADSVTG

SEQ ID NO: 41 - protein, 17 aa, synthetic construct
CISSSDASTYYADSVKG

SEQ ID NO: 42 - protein, 17 aa, synthetic construct
CISSSEGSTYYADSVKG

SEQ ID NO: 43 - protein, 17 aa, synthetic construct
CISSSDASTYYADSVKG

SEQ ID NO: 44 - protein, 17 aa, synthetic construct
CISSSEGSTYYADSVKG